European Patent Specification EP 3 722 431 B1, published June 10, 2026. Title: SECRETION OF HEME-CONTAINING POLYPEPTIDES. Applicant: Impossible Foods Inc. The sequence listing filed with the application follows.

SEQUENCE LISTING (96 sequences)

SEQ ID NO: 1 - protein, 161 aa, Vigna radiata
MTTTLERGFTEEQEALVVKSWNVMKKNSGELGLKFFLKIFEIAPSAQKLFSFLRDSTVPLEQNPKLKPHAVSVFVMTCDSAVQLRKAGKVTVRESNLKKLGATHFRTGVANEHFEVTKFALLETIKEAVPEMWSPAMKNAWGEAYDQLVDAIKYEMKPPSS

SEQ ID NO: 2 - protein, 133 aa, Methylacidiphilum infernorum
MIDQKEKELIKESWKRIEPNKNEIGLLFYANLFKEEPTVSVLFQNPISSQSRKLMQVLGILVQGIDNLEGLIPTLQDLGRRHKQYGVVDSHYPLVGDCLLKSIQEYLGQGFTEEAKAAWTKVYGIAAQVMTAE

SEQ ID NO: 3 - protein, 139 aa, Aquifex aeolicus
MLSEETIRVIKSTVPLLKEHGTEITARMYELLFSKYPKTKELFAGASEEQPKKLANAIIAYATYIDRLEELDNAISTIARSHVRRNVKPEHYPLVKECLLQAIEEVLNPGEEVLKAWEEAYDFLAKTLITLEKKLYSQP

SEQ ID NO: 4 - protein, 145 aa, Glycine max
MGAFTEKQEALVSSSFEAFKANIPQYSVVFYTSILEKAPAAKDLFSFLSNGVDPSNPKLTGHAEKLFGLVRDSAGQLKANGTVVADAALGSIHAQKAITDPQFVVVKEALLKTIKEAVGDKWSDELSSAWEVAYDELAAAIKKAF

SEQ ID NO: 5 - protein, 162 aa, Hordeum vulgare
MSAAEGAVVFSEEKEALVLKSWAIMKKDSANLGLRFFLKIFEIAPSARQMFPFLRDSDVPLETNPKLKTHAVSVFVMTCEAAAQLRKAGKITVRETTLKRLGGTHLKYGVADGHFEVTRFALLETIKEALPADMWGPEMRNAWGEAYDQLVAAIKQEMKPAE

SEQ ID NO: 6 - protein, 1153 aa, Magnaporthe oryzae
MDGAVRLDWTGLDLTGHEIHDGVPIASRVQVMVSFPLFKDQHIIMSSKESPSRKSSTIGQSTRNGSCQADTQKGQLPPVGEKPKPVKENPMKKLKEMSQRPLPTQHGDGTYPTEKKLTGIGEDLKHIRGYDVKTLLAMVKSKLKGEKLKDDKTMLMERVMQLVARLPTESKKRAELTDSLINELWESLDHPPLNYLGPEHSYRTPDGSYNHPFNPQLGAAGSRYARSVIPTVTPPGALPDPGLIFDSIMGRTPNSYRKHPNNVSSILWYWATIIIHDIFWTDPRDINTNKSSSYLDLAPLYGNSQEMQDSIRTFKDGRMKPDCYADKRLAGMPPGVSVLLIMFNRFHNHVAENLALINEGGRFNKPSDLLEGEAREAAWKKYDNDLFQVARLVTSGLYINITLVDYVRNIVNLNRVDTTWTLDPRQDAGAHVGTADGAERGTGNAVSAEFNLCYRWHSCISEKDSKFVEAQFQNIFGKPASEVRPDEMWKGFAKMEQNTPADPGQRTFGGFKRGPDGKFDDDDLVRCISEAVEDVAGAFGARNVPQAMKVVETMGIIQGRKWNVAGLNEFRKHFHLKPYSTFEDINSDPGVAEALRRLYDHPDNVELYPGLVAEEDKQPMVPGVGIAPTYTISRVVLSDAVCLVRGDRFYTTDFTPRNLTNWGYKEVDYDLSVNHGCVFYKLFIRAFPNHFKQNSVYAHYPMVVPSENKRILEALGRADLFDFEAPKYIPPRVNITSYGGAEYILETQEKYKVTWHEGLGFLMGEGGLKFMLSGDDPLHAQQRKCMAAQLYKDGWTEAVKAFYAGMMEELLVSKSYFLGNNKHRHVDIIRDVGNMVHVHFASQVFGLPLKTAKNPTGVFTEQEMYGILAAIFTTIFFDLDPSKSFPLRTKTREVCQKLAKLVEANVKLINKIPWSRGMFVGKPAKDEPLSIYGKTMIKGLKAHGLSDYDIAWSHVVPTSGAMVPNQAQVFAQAVDYYLSPAGMHYIPEIHMVALQPSTPETDALLLGYAMEGIRLAGTFGSYREAAVDDVVKEDNGRQVPVKAGDRVFVSFVDAARDPKHFPDPEVVNPRRPAKKYIHYGVGPHACLGRDASQIAITEMFRCLFRRRNVRRVPGPQGELKKVPRPGGFYVYMREDWGGLFPFPVTMRVMWDDE

SEQ ID NO: 7 - protein, 530 aa, Fusarium oxysporum
MKGSATLAFALVQFSAASQLVWPSKWDEVEDLLYMQGGFNKRGFADALRTCEFGSNVPGTQNTAEWLRTAFHDAITHDAKAGTGGLDASIYWESSRPENPGKAFNNTFGFFSGFHNPRATASDLTALGTVLAVGACNGPRIPFRAGRIDAYKAGPAGVPEPSTNLKDTFAAFTKAGFTKEEMTAMVACGHAIGGVHSVDFPEIVGIKADPNNDTNVPFQKDVSSFHNGIVTEYLAGTSKNPLVASKNATFHSDKRIFDNDKATMKKLSTKAGFNSMCADILTRMIDTVPKSVQLTPVLEAYDVRPYITELSLNNKNKIHFTGSVRVRITNNIRDNNDLAINLIYVGRDGKKVTVPTQQVTFQGGTSFGAGEVFANFEFDTTMDAKNGITKFFIQEVKPSTKATVTHDNQKTGGYKVDDTVLYQLQQSCAVLEKLPNAPLVVTAMVRDARAKDALTLRVAHKKPVKGSIVPRFQTAITNFKATGKKSSGYTGFQAKTMFEEQSTYFDIVLGGSPASGVQFLTSQAMPSQCS

SEQ ID NO: 8 - protein, 358 aa, Fusarium graminearum
MASATRQFARAATRATRNGFAIAPRQVIRQQGRRYYSSEPAQKSSSAWIWLTGAAVAGGAGYYFYGNSASSATAKVFNPSKEDYQKVYNEIAARLEEKDDYDDGSYGPVLVRLAWHASGTYDKETGTGGSNGATMRFAPESDHGANAGLAAARDFLQPVKEKFPWITYSDLWILAGVCAIQEMLGPAIPYRPGRSDRDVSGCTPDGRLPDASKRQDHLRGIFGRMGFNDQEIVALSGAHALGRCHTDRSGYSGPWTFSPTVLTNDYFRLLVEEKWQWKKWNGPAQYEDKSTKSLMMLPSDIALIEDKKFKPWVEKYAKDNDAFFKDFSNVVLRLFELGVPFAQGTENQRWTFKPTHQE

SEQ ID NO: 9 - protein, 122 aa, Chlamydomonas eugametos
MSLFAKLGGREAVEAAVDKFYNKIVADPTVSTYFSNTDMKVQRSKQFAFLAYALGGASEWKGKDMRTAHKDLVPHLSDVHFQAVARHLSDTLTELGVPPEDITDAMAVVASTRTEVLNMPQQ

SEQ ID NO: 10 - protein, 121 aa, Tetrahymena pyriformis
MNKPQTIYEKLGGENAMKAAVPLFYKKVLADERVKHFFKNTDMDHQTKQQTDFLTMLLGGPNHYKGKNMTEAHKGMNLQNLHFDAIIENLAATLKELGVTDAVINEAAKVIEHTRKDMLGK

SEQ ID NO: 11 - protein, 117 aa, Paramecium caudatum
MSLFEQLGGQAAVQAVTAQFYANIQADATVATFFNGIDMPNQTNKTAAFLCAALGGPNAWTGRNLKEVHANMGVSNAQFTTVIGHLRSALTGAGVAAALVEQTVAVAETVRGDVVTV

SEQ ID NO: 12 - protein, 147 aa, Aspergillus niger
MPLTPEQIKIIKATVPVLQEYGTKITTAFYMNMSTVHPELNAVFNTANQVKGHQARALAGALFAYASHIDDLGALGPAVELICNKHASLYIQADEYKIVGKYLLEAMKEVLGDACTDDILDAWGAAYWALADIMINREAALYKQSQG

SEQ ID NO: 13 - protein, 165 aa, Zea mays
MALAEADDGAVVFGEEQEALVLKSWAVMKKDAANLGLRFFLKVFEIAPSAEQMFSFLRDSDVPLEKNPKLKTHAMSVFVMTCEAAAQLRKAGKVTVRETTLKRLGATHLRYGVADGHFEVTGFALLETIKEALPADMWSLEMKKAWAEAYSQLVAAIKREMKPDA

SEQ ID NO: 14 - protein, 169 aa, Oryza sativa subsp. japonica
MALVEGNNGVSGGAVSFSEEQEALVLKSWAIMKKDSANIGLRFFLKIFEVAPSASQMFSFLRNSDVPLEKNPKLKTHAMSVFVMTCEAAAQLRKAGKVTVRDTTLKRLGATHFKYGVGDAHFEVTRFALLETIKEAVPVDMWSPAMKSAWSEAYNQLVAAIKQEMKPAE

SEQ ID NO: 15 - protein, 160 aa, Arabidopsis thaliana
MESEGKIVFTEEQEALVVKSWSVMKKNSAELGLKLFIKIFEIAPTTKKMFSFLRDSPIPAEQNPKLKPHAMSVFVMCCESAVQLRKTGKVTVRETTLKRLGASHSKYGVVDEHFEVAKYALLETIKEAVPEMWSPEMKVAWGQAYDHLVAAIKAEMNLSN

SEQ ID NO: 16 - protein, 147 aa, Pisum sativum
MGFTDKQEALVNSSWESFKQNLSGNSILFYTIILEKAPAAKGLFSFLKDTAGVEDSPKLQAHAEQVFGLVRDSAAQLRTKGEVVLGNATLGAIHVQRGVTDPHFVVVKEALLQTIKKASGNNWSEELNTAWEVAYDGLATAIKKAMT

SEQ ID NO: 17 - protein, 145 aa, Vigna unguiculata
MVAFSDKQEALVNGAYEAFKANIPKYSVVFYTTILEKAPAAKNLFSFLANGVDATNPKLTGHAEKLFGLVRDSAAQLRASGGVVADAALGAVHSQKAVNDAQFVVVKEALVKTLKEAVGDKWSDELGTAVELAYDELAAAIKKAY

SEQ ID NO: 18 - protein, 154 aa, Bos taurus
MGLSDGEWQLVLNAWGKVEADVAGHGQEVLIRLFTGHPETLEKFDKFKHLKTEAEMKASEDLKKHGNTVLTALGGILKKKGHHEAEVKHLAESHANKHKIPVKYLEFISDAIIHVLHAKHPSDFGADAQAAMSKALELFRNDMAAQYKVLGFHG

SEQ ID NO: 19 - protein, 154 aa, Sus scrofa
MGLSDGEWQLVLNVWGKVEADVAGHGQEVLIRLFKGHPETLEKFDKFKHLKSEDEMKASEDLKKHGNTVLTALGGILKKKGHHEAELTPLAQSHATKHKIPVKYLEFISEAIIQVLQSKHPGDFGADAQGAMSKALELFRNDMAAKYKELGFQG

SEQ ID NO: 20 - protein, 154 aa, Equus caballus
MGLSDGEWQQVLNVWGKVEADIAGHGQEVLIRLFTGHPETLEKFDKFKHLKTEAEMKASEDLKKHGTVVLTALGGILKKKGHHEAELKPLAQSHATKHKIPIKYLEFISDAIIHVLHSKHPGDFGADAQGAMTKALELFRNDIAAKYKELGFQG

SEQ ID NO: 21 - protein, 124 aa, Synechocystis PCC6803
MSTLYEKLGGTTAVDLAVDKFYERVLQDDRIKHFFADVDMAKQRAHQKAFLTYAFGGTDKYDGRYMREAHKELVENHGLNGEHFDAVAEDLLATLKEMGVPEDLIAEVAAVAGAPAHKRDVLNQ

SEQ ID NO: 22 - protein, 183 aa, Synechococcus sp. PCC 7335
MDVALLEKSFEQISPRAIEFSASFYQNLFHHHPELKPLFAETSQTIQEKKLIFSLAAIIENLRNPDILQPALKSLGARHAEVGTIKSHYPLVGQALIETFAEYLAADWTEQLATAWVEAYDVIASTMIEGADNPAAYLEPELTFYEWLDLYGEESPKVRNAIATLTHFHYGEDPQDVQRDSRG

SEQ ID NO: 23 - protein, 118 aa, Nostoc commune
MSTLYDNIGGQPAIEQVVDELHKRIATDSLLAPVFAGTDMVKQRNHLVAFLAQIFEGPKQYGGRPMDKTHAGLNLQQPHFDAIAKHLGERMAVRGVSAENTKAALDRVTNMKGAILNK

SEQ ID NO: 24 - protein, 146 aa, Vitreoscilla stercoraria
MLDQQTINIIKATVPVLKEHGVTITTTFYKNLFAKHPEVRPLFDMGRQESLEQPKALAMTVLAAAQNIENLPAILPAVKKIAVKHCQAGVAAAHYPIVGQELLGAIKEVLGDAATDDILDAWGKAYGVIADVFIQVEADLYAQAVE

SEQ ID NO: 25 - protein, 131 aa, Corynebacterium glutamicum
MTTSENFYDSVGGEETFSLIVHRFYEQVPNDDILGPMYPPDDFEGAEQRLKMFLSQYWGGPKDYQEQRGHPRLRMRHVNYPIGVTAAERWLQLMSNALDGVDLTAEQREAIWEHMVRAADMLINSNPDPHA

SEQ ID NO: 26 - protein, 132 aa, Bacillus subtilis
MGQSFNAPYEAIGEELLSQLVDTFYERVASHPLLKPIFPSDLTETARKQKQFLTQYLGGPPLYTEEHGHPMLRARHLPFPITNERADAWLSCMKDAMDHVGLEGEIREFLFGRLELTARHMVNQTEAEDRSS

SEQ ID NO: 27 - protein, 136 aa, Bacillus megaterium
MREKIHSPYELLGGEHTISKLVDAFYTRVGQHPELAPIFPDNLTETARKQKQFLTQYLGGPSLYTEEHGHPMLRARHLPFEITPSRAKAWLTCMHEAMDEINLEGPERDELYHRLILTAQHMINSPEQTDEKGFSH

SEQ ID NO: 28 - protein, 399 aa, Saccharomyces cerevisiae [sequence omitted]

SEQ ID NO: 29 - protein, 152 aa, Nicotina tobaccum
MSSFSEEQEALVLKSWDSMKKNAGEWGLKLFLKIFEIAPSAKKLFSFLKDSNVPLEQNAKLKPHAKSVFVMTCEAAVQLRKAGKVVVRDSTLKKLGAAHFKYGVADEHFEVTKFALLETIKEAVPDMWSVDMKNAWGEAFDQLVNAIKTEMK

SEQ ID NO: 30 - protein, 160 aa, Medicago sativa
MGTLDTKGFTEEQEALVVKSWNAMKKNSAELGLKLFLKIFEIAPSAQKLFSFLKDSKVPLEQNTKLKPHAMSVFLMTCESAVQLRKSGKVTVRESSLKKLGANHFKYGVVDEHFEVTKFALLETIKEAVPEMWSPAMKNAWGEAYDQLVNAIKSEMKPSS

SEQ ID NO: 31 - protein, 161 aa, Glycine max
MTTTLERGFSEEQEALVVKSWNVMKKNSGELGLKFFLKIFEIAPSAQKLFSFLRDSTVPLEQNPKLKPHAVSVFVMTCDSAVQLRKAGKVTVRESNLKKLGATHFRTGVANEHFEVTKFALLETIKEAVPEMWSPAMKNAWGEAYDQLVDAIKSEMKPPSS

SEQ ID NO: 32 - DNA, 97 bp, Artificial Sequence
  encodes signal peptide
atgaaaaagaaaaaaacatggaaacgcttcttacacttttcgagtgcagctctggctgcaggtttgatattcacttctgctgctcccgcagaggcag

SEQ ID NO: 33 - protein, 33 aa, Artificial Sequence
  signal peptide
MKKKKTWKRFLHFSSAALAAGLIFTSAAPAEAA

SEQ ID NO: 34 - DNA, 131 bp, Artificial Sequence
  encodes signal peptide
atgtcaccagcacaaagaagaattttactgtatatcctttcatttatctttgtcatcggcgcagtcgtctattttgtcaaaagcgattatctgtttacgctgattttcattgccattgccattctgttcgg

SEQ ID NO: 35 - protein, 43 aa, Artificial Sequence
  signal peptide
MSPAQRRILLYILSFIFVIGAVVYFVKSDYLFTLIFIAIAILF

SEQ ID NO: 36 - DNA, 90 bp, Artificial Sequence
  encodes signal peptide
atggtcagcatccgccgcagcttcgaagcgtatgtcgatgacatgaatatcattactgttctgattcctgctgaacaaaaggaaatcatg

SEQ ID NO: 37 - protein, 30 aa, Artificial Sequence
  signal peptide
MVSIRRSFEAYVDDMNIITVLIPAEQKEIM

SEQ ID NO: 38 - DNA, 99 bp, Artificial Sequence
  encodes signal peptide
atggctgcatatattatcagaagaaccttaatgtctatcccgattttattgggaattacgattttatcatttgttatcatgaaagccgcgcccggagat

SEQ ID NO: 39 - protein, 33 aa, Artificial Sequence
  signal peptide
MAAYIIRRTLMSIPILLGITILSFVIMKAAPGD

SEQ ID NO: 40 - DNA, 87 bp, Artificial Sequence
  encodes signal peptide
atgaaacggtcaatctctatttttattacgtgtttattgattacgttattgacaatgggcggcatgatagcttcgccggcatcagca

SEQ ID NO: 41 - protein, 29 aa, Artificial Sequence
  signal peptide
MKRSISIFITCLLITLLTMGGMIASPASA

SEQ ID NO: 42 - DNA, 93 bp, Artificial Sequence
  encodes signal peptide
atgccttatctgaaacgagtgttgctgcttcttgtcactggattgtttatgagtttgtttgcagtcactgctactgcctcagctcaaacaggt

SEQ ID NO: 43 - protein, 31 aa, Artificial Sequence
  signal peptide
MPYLKRVLLLLVTGLFMSLFAVTATASAQTG

SEQ ID NO: 44 - DNA, 102 bp, Artificial Sequence
  encodes signal peptide
atgaaatttgtaaaaagaaggatcattgcacttgtaacaattttgatgctgtctgttacatcgctgtttgcgttgcagccgtcagcaaaagccgctgaacac

SEQ ID NO: 45 - protein, 34 aa, Artificial Sequence
  signal peptide
MKFVKRRIIALVTILMLSVTSLFALQPSAKAAEH

SEQ ID NO: 46 - DNA, 90 bp, Artificial Sequence
  encodes signal peptide
atgaaaaagagactaatcgcacctatgcttctatccgccgcgtcccttgccttttttgccatgtctggttctgcccaggcagccgcgtat

SEQ ID NO: 47 - protein, 30 aa, Artificial Sequence
  signal peptide
MKKRLIAPMLLSAASLAFFAMSGSAQAAAY

SEQ ID NO: 48 - DNA, 72 bp, Artificial Sequence
  encodes signal peptide
atgaaaaaacgttggtcgattgtcacgttgatgctcattttcactctcgtgctgagcgcgtgcggctttggc

SEQ ID NO: 49 - protein, 24 aa, Artificial Sequence
  signal peptide
MKKRWSIVTLMLIFTLVLSACGFG

SEQ ID NO: 50 - DNA, 99 bp, Artificial Sequence
  encodes signal peptide
atgctaaaatatatcggaagacgcttagtctatatgattatcacactatttgtgattgtaactgtgacattcttcttaatgcaagcagcaccgggcggg

SEQ ID NO: 51 - protein, 33 aa, Artificial Sequence
  signal peptide
MLKYIGRRLVYMIITLFVIVTVTFFLMQAAPGG

SEQ ID NO: 52 - DNA, 126 bp, Artificial Sequence
  encodes signal peptide
atgacaagcccaacccgcagaagaactgcgaaacgcagacggagaaaactaaataaaagaggaaaactgttgtttggtcttttagcagtgatggtttgcattacgatttggaatgctcttcatcga

SEQ ID NO: 53 - protein, 42 aa, Artificial Sequence
  signal peptide
MTSPTRRRTAKRRRRKLNKRGKLLFGLLAVMVCITIWNALHR

SEQ ID NO: 54 - DNA, 168 bp, Artificial Sequence
  encodes signal peptide
atggcatacgacagtcgttttgatgaatgggtacagaaactgaaagaggaaagctttcaaaacaatacgtttgaccgccgcaaatttattcaaggagcggggaagattgcaggactttctcttggattaacgattgcccagtcggttggggcctttgaagtaaatgct

SEQ ID NO: 55 - protein, 56 aa, Artificial Sequence
  signal peptide
MAYDSRFDEWVQKLKEESFQNNTFDRRKFIQGAGKIAGLSLGLTIAQSVGAFEVNA

SEQ ID NO: 56 - DNA, 117 bp, Artificial Sequence
  encodes signal peptide
atgggcggaaaacatgatatatccagacgtcaatttttgaattatacgctcacaggcgtaggaggttttatggcggctagtatgctcatgcctatggttcgcttcgcactcgacccg

SEQ ID NO: 57 - protein, 39 aa, Artificial Sequence
  signal peptide
MGGKHDISRRQFLNYTLTGVGGFMAASMLMPMVRFALDP

SEQ ID NO: 58 - DNA, 78 bp, Artificial Sequence
  encodes signal peptide
atgttgttgaaaaggagaatagggttgctattaagtatggttggcgtattcatgcttttggctggatgctcgagtgtg

SEQ ID NO: 59 - protein, 26 aa, Artificial Sequence
  signal peptide
MLLKRRIGLLLSMVGVFMLLAGCSSV

SEQ ID NO: 60 - DNA, 129 bp, Artificial Sequence
  encodes signal peptide
atgaaaaaaacactcaccactattcgcagatcatcaattgcaaggagacttattatttctttcctgctgatcttaattgttccgataaccgccctttcggttagcgcttatcaatcagcagttgcctca

SEQ ID NO: 61 - protein, 43 aa, Artificial Sequence
  signal peptide
MKKTLTTIRRSSIARRLIISFLLILIVPITALSVSAYQSAVAS

SEQ ID NO: 62 - DNA, 105 bp, Artificial Sequence
  encodes signal peptide
atgaaaaaaagaaagaggcgaaactttaaaaggttcattgcagcatttttagtgttggctttaatgatttcattagtgccagccgatgtactagcaaaatctaca

SEQ ID NO: 63 - protein, 35 aa, Artificial Sequence
  signal peptide
MKKRKRRNFKRFIAAFLVLALMISLVPADVLAKST

SEQ ID NO: 64 - DNA, 102 bp, Artificial Sequence
  encodes signal peptide
atgaaacgcagaaaattcagctcggttgtggcggcagtgcttatttttgcactgattttcagccttttttctccgggaaccaaagctgcagcggccggcgcg

SEQ ID NO: 65 - protein, 34 aa, Artificial Sequence
  signal peptide
MKRRKFSSVVAAVLIFALIFSLFSPGTKAAAAGA

SEQ ID NO: 66 - DNA, 78 bp, Artificial Sequence
  encodes signal peptide
atgaagaaacgcagaaagatatgttattgcaatactgccctgctgcttatgattttgcttgctggatgtacggacagt

SEQ ID NO: 67 - protein, 26 aa, Artificial Sequence
  signal peptide
MKKRRKICYCNTALLLMILLAGCTDS

SEQ ID NO: 68 - DNA, 129 bp, Artificial Sequence
  encodes signal peptide
atgaagaaaagagttgctggctggtacaggcggatgaagattaaggataagctgtttgtgtttctatcgttgattatggccgtatcctttctgtttgtatacagcggggtccagtatgcctttcatgtg

SEQ ID NO: 69 - protein, 43 aa, Artificial Sequence
  signal peptide
MKKRVAGWYRRMKIKDKLFVFLSLIMAVSFLFVYSGVQYAFHV

SEQ ID NO: 70 - DNA, 114 bp, Artificial Sequence
  encodes signal peptide
atgagaaggagctgtctgatgattagacgaaggaaacgcatgtttaccgctgttacgttgctggtcttgttggtgatgggaacctctgtatgtcctgtgaaagctgaaggggca

SEQ ID NO: 71 - protein, 38 aa, Artificial Sequence
  signal peptide
MRRSCLMIRRRKRMFTAVTLLVLLVMGTSVCPVKAEGA

SEQ ID NO: 72 - DNA, 114 bp, Artificial Sequence
  encodes signal peptide
atgagaatacagaaaagacgaacacacgtcgaaaacattctccgtattcttttgcccccaattatgatacttagcctaatcctcccaacaccacccattcatgcagaagaaagc

SEQ ID NO: 73 - protein, 38 aa, Artificial Sequence
  signal peptide
MRIQKRRTHVENILRILLPPIMILSLILPTPPIHAEES

SEQ ID NO: 74 - DNA, 147 bp, Artificial Sequence
  encodes signal peptide
atgctgtctgtcgaaatgataagcagacaaaatcgttgtcattatgtgtataagggaggaaatatgatgaggcgtattctgcatattgtgttgatcacggcattaatgttcttaaatgtaatgtacacgttcgaagctgtaaaggca

SEQ ID NO: 75 - protein, 49 aa, Artificial Sequence
  signal peptide
MLSVEMISRQNRCHYVYKGGNMMRRILHIVLITALMFLNVMYTFEAVKA

SEQ ID NO: 76 - DNA, 93 bp, Artificial Sequence
  encodes signal peptide
atgctaagagatttaggaagaagagtagcgatcgcagccattttaagcggaattattcttggaggcatgagcatttctttggcaaatatgccc

SEQ ID NO: 77 - protein, 31 aa, Artificial Sequence
  signal peptide
MLRDLGRRVAIAAILSGIILGGMSISLANMP

SEQ ID NO: 78 - DNA, 102 bp, Artificial Sequence
  encodes signal peptide
atgaaaaagatgtccagaagacaatttctaaaaggaatgttcggcgctcttgctgccggggctttaacggccggcgggggatatggctatgccaggtatctc

SEQ ID NO: 79 - protein, 34 aa, Artificial Sequence
  signal peptide
MKKMSRRQFLKGMFGALAAGALTAGGGYGYARYL

SEQ ID NO: 80 - DNA, 84 bp, Artificial Sequence
  encodes signal peptide
atgagaagatttttactaaatgtcatattagtcttagccattgtcttgttcttgagatatgttcattactcattggaaccagaa

SEQ ID NO: 81 - protein, 28 aa, Artificial Sequence
  signal peptide
MRRFLLNVILVLAIVLFLRYVHYSLEPE

SEQ ID NO: 82 - DNA, 87 bp, Artificial Sequence
  encodes signal peptide
atgtttgaaagtgaagcagaactgagacgaatcaggattgcacttgtatggatagctgtctttttactgttcggggcgtgcgggaat

SEQ ID NO: 83 - protein, 29 aa, Artificial Sequence
  signal peptide
MFESEAELRRIRIALVWIAVFLLFGACGN

SEQ ID NO: 84 - DNA, 93 bp, Artificial Sequence
  encodes signal peptide
atgaagaagagaattacatattcactgcttgctcttctagcagttgttgctttcgctttcactgattcatcaaaagcaaaagcggcagaagca

SEQ ID NO: 85 - protein, 31 aa, Artificial Sequence
  signal peptide
MKKRITYSLLALLAVVAFAFTDSSKAKAAEA

SEQ ID NO: 86 - DNA, 116 bp, Artificial Sequence
  encodes signal peptide
atgcagaaatatagacgcagaaacacggttgcctttacagtactagcttattttactttttttgcgggagtatttttgtttagtatcggactctataatgctgataatctggaact

SEQ ID NO: 87 - protein, 38 aa, Artificial Sequence
  signal peptide
MQKYRRRNTVAFTVLAYFTFFAGVFLFSIGLYNADNLE

SEQ ID NO: 88 - DNA, 102 bp, Artificial Sequence
  encodes signal peptide
atgatgttgaatatgatcagacgtttgctgatgacctgtttatttctgcttgcatttggcacgacatttttatcagtgtcaggaattgaagcgaaggacttg

SEQ ID NO: 89 - protein, 34 aa, Artificial Sequence
  signal peptide
MMLNMIRRLLMTCLFLLAFGTTFLSVSGIEAKDL

SEQ ID NO: 90 - DNA, 132 bp, Artificial Sequence
  encodes signal peptide
atggctgaacgcgttagagtgcgtgtgcgaaaaaagaaaaagagcaaacgtaggaaaattttaaaaagaataatgttattgttcgcccttgcactattggtagttgtagggcttggcgggtataaactttat

SEQ ID NO: 91 - protein, 44 aa, Artificial Sequence
  signal peptide
MAERVRVRVRKKKKSKRRKILKRIMLLFALALLVVVGLGGYKLY

SEQ ID NO: 92 - DNA, 141 bp, Artificial Sequence
  encodes signal peptide
atgagcgatgaacagaaaaagccagaacaaattcacagacgggacattttaaaatggggagcgatggcgggggcagccgttgcgatcggtgccagcggtctcggcggtctcgctccgcttgttcagactgcggctaagcca

SEQ ID NO: 93 - protein, 47 aa, Artificial Sequence
  signal peptide
MSDEQKKPEQIHRRDILKWGAMAGAAVAIGASGLGGLAPLVQTAAKP

SEQ ID NO: 94 - protein, 204 aa, Artificial Sequence
  fusion protein
MAYDSRFDEWVQKLKEESFQNNTFDRRKFIQGAGKIAGLSLGLTIAQSASAAGAHMELGLSEETIRVIKSTVPLLKEHGTEITARMYELLFSKYPKTKELFAGASEEQPKKLANAIIAYATYIDRLEELDNAISTIARSHVRRNVKPEHYPLVKECLLQAIEEVLNPGEEVLKAWEEAYDFLAKTLITLEKKLYSQPRHHHHHH

SEQ ID NO: 95 - protein, 156 aa, Artificial Sequence
  signal peptidase I recognition site
ASAAGAHMELGLSEETIRVIKSTVPLLKEHGTEITARMYELLFSKYPKTKELFAGASEEQPKKLANAIIAYATYIDRLEELDNAISTIARSHVRRNVKPEHYPLVKECLLQAIEEVLNPGEEVLKAWEEAYDFLAKTLITLEKKLYSQPRHHHHHH

SEQ ID NO: 96 - protein, 10 aa, Artificial Sequence
  N-terminal peptide
GAHMELGLSE